European Patent Application EP 4 772 641 A1, published July 8, 2026. Title: A novel promoter and method for producing L-lysine using thereof. Applicant: CJ CheilJedang Corporation. The sequence listing filed with the application follows.

SEQUENCE LISTING (67 sequences)

SEQ ID NO: 1 - DNA, 170 bp, synthetic construct
  misc_feature 1..170: note = Promoter variant of NCgl0302 gene
  source 1..170: mol_type = other DNA
actgcgcactgaaactgcggcctgggaacaagtctttcacgtttaaagcccaagcgatagtctattaggattagttttacgttttggcaggtcagtcccatttatacagcccagcgaaagggggtaaattcttgactacccccgattttgagagtgaaaagactcaagct

SEQ ID NO: 2 - DNA, 220 bp, synthetic construct
  misc_feature 1..220: note = Promoter variant of NCgl0123 gene
  source 1..220: mol_type = other DNA
actttcacatcaaaaaaagggggacaaatttctacatgaaattcgacgagatgaatgctattcattcttgtcttcagccacatctattcgaaatgaaatcctactgaatcaccagctagtccgcctaggtaaaaaaggcgtaattaacttatttatacataaaaacacaataaaaaccgcacacgcggcgaaacttcaataaatccctagactgcaaaaa

SEQ ID NO: 3 - DNA, 215 bp, synthetic construct
  misc_feature 1..215: note = Promoter variant of NCgl0625 gene
  source 1..215: mol_type = other DNA
gagagatgatttataccatcctacaccatttagagtggggctagtcatacccccataaccctagctgtacgcaatcgatttcaaatcagttggaaaaagtcaagaaaattacccgagaataaatttataccacacagtctattgcaatagaccaagctgttcagtagggtgcatgggagaagaatttcctaataaaaactcttaaggacctccaa

SEQ ID NO: 4 - DNA, 190 bp, synthetic construct
  misc_feature 1..190: note = Promoter variant of NCgl0276 gene
  source 1..190: mol_type = other DNA
ggcgcaccccaggcgcaccccaggcgcaccccagcgcaccacaggcgcaccccagcgcaccacaggcgcaccccagcgcaccacaggcgcaccagcccagcacaagagccaacgcaagtgtcaggcacgccagcaaaggggctagcaagaagcacgcccccgaagccttagaaatgcgttccccggtagg

SEQ ID NO: 5 - DNA, 63 bp, synthetic construct
  misc_feature 1..63: note = Promoter variant of NCgl1064 gene
  source 1..63: mol_type = other DNA
cattttcatatgttaatcgaccgcttccatcatgttttaactaaggtttgtaggcttaaacct

SEQ ID NO: 6 - DNA, 308 bp, synthetic construct
  misc_feature 1..308: note = Promoter variant of NCgl0294 gene
  source 1..308: mol_type = other DNA
gcgcctcggggggggggtgtgcgcgggccgtcagtaacccggcaacggggggggattgtgccggggcaggccacactgtatatcggggccttgcacctgaaattatggcatatcaaacgccacaagacaacatcaaacccgattatttattcgaataacacgaatacttaacagtgtggcaaatgacacttcccgcacgccttctacattcccaatgcgcaaccccagcacgtcacttcaatctcattggtaactttagtttctttctcagtcttggaaagttgccaaaaagcgctaaactatgcggt

SEQ ID NO: 7 - DNA, 225 bp, synthetic construct
  misc_feature 1..225: note = Promoter variant of NCgl1720 gene
  source 1..225: mol_type = other DNA
gcggttgattaaaaaaaagaacactttgatatgaattaagtcgaagtgttcttttattaatttaaaagtatatttcagcaatggtaaatgaatctcataagttttaaagaaaagtattgcatttgtttgacaaggtgattatgcttcacattaatacttaataagaattgttctgggaagtaatataaaaagtcccgaacaaattagtgtgaaagggtttgtatc

SEQ ID NO: 8 - DNA, 246 bp, synthetic construct
  misc_feature 1..246: note = Promoter variant of NCgl0246 gene
  source 1..246: mol_type = other DNA
ctttgtgcacctttcgatctaggtgctgacagttacccgctcaactctacctttataaactgtgtctacctagccagaggagtgttttctttctgcacagggttcctggggctttagcggatgcgtctcagccactgggacgcgttccaataaacagaccatatattgatattcgatttaatatttgagacaaaagtgacaggtgctacttcgcgagcaactctttagtcaactaccctgaatcaa

SEQ ID NO: 9 - DNA, 164 bp, synthetic construct
  misc_feature 1..164: note = Promoter variant of NCgl2356 gene
  source 1..164: mol_type = other DNA
agattttgcttttcgacgctcccctccacctcattcaatgcggcgggaggggatttccttgcatgttaagcctataggaaaaagtgtttgcatatcacccttgtattcgaacacgtgagcgggtagagtgggtggtaacaacacggggaaagggggaagacacc

SEQ ID NO: 10 - DNA, 198 bp, synthetic construct
  misc_feature 1..198: note = Promoter variant of NCgl2521 gene
  source 1..198: mol_type = other DNA
gacgggctgaaaccaaaccagactgcccggcaacgacggaaatcccaaaagtgggcatccctgtttggtaccgagtacccacccgggcctgaaactccctggcaggcgggcgaagcgtggcaacaactggaatttaagagcacaattgaagtcgcaccaagttaggcaacacaatagccataacgttgaggagttcag

SEQ ID NO: 11 - DNA, 210 bp, synthetic construct
  misc_feature 1..210: note = Promoter variant of NCgl2960 gene
  source 1..210: mol_type = other DNA
cctcaatgtcacgtgaaacattgagggttttacacccaattaagaaaaaatgaattaaaccaaaacttcttaatcgcaggggttaaggtaagttcagctaatcaatgaaacttcccctttcagcccgttgaagaaccaatgagccctgcccgcacccagccccgagcggctttcctaaggaagctccgacccatcacatgtagcctttcc

SEQ ID NO: 12 - DNA, 40 bp, synthetic construct
  misc_feature 1..40: note = Pn*_NCgl0302_F
  source 1..40: mol_type = other DNA
tgaattcgagctcggtacccgccgatttcgaactcgacga

SEQ ID NO: 13 - DNA, 40 bp, synthetic construct
  misc_feature 1..40: note = Pn*_NCgl0302_R
  source 1..40: mol_type = other DNA
gtcgactctagaggatcccccacatgctggccattccacg

SEQ ID NO: 14 - DNA, 40 bp, synthetic construct
  misc_feature 1..40: note = Pn*_NCgl0123_F
  source 1..40: mol_type = other DNA
tgaattcgagctcggtaccctgtgtgctcgggaatcatta

SEQ ID NO: 15 - DNA, 40 bp, synthetic construct
  misc_feature 1..40: note = Pn*_NCgl0123_R
  source 1..40: mol_type = other DNA
gtcgactctagaggatccccaggcggcttttacggcgcgg

SEQ ID NO: 16 - DNA, 40 bp, synthetic construct
  misc_feature 1..40: note = Pn*_NCgl0625_F
  source 1..40: mol_type = other DNA
tgaattcgagctcggtacccaagtgcgaaacgctgcttgg

SEQ ID NO: 17 - DNA, 40 bp, synthetic construct
  misc_feature 1..40: note = Pn*_NCgl0625_R
  source 1..40: mol_type = other DNA
gtcgactctagaggatccccaacgcgggcggtcggtgaca

SEQ ID NO: 18 - DNA, 40 bp, synthetic construct
  misc_feature 1..40: note = Pn*_NCgl0276_F
  source 1..40: mol_type = other DNA
tgaattcgagctcggtacccgcagcagcaatttgccgcca

SEQ ID NO: 19 - DNA, 40 bp, synthetic construct
  misc_feature 1..40: note = Pn*_NCgl0276_R
  source 1..40: mol_type = other DNA
gtcgactctagaggatccccggcagctgaccagaagtcca

SEQ ID NO: 20 - DNA, 40 bp, synthetic construct
  misc_feature 1..40: note = Pn*_NCgl1064_F
  source 1..40: mol_type = other DNA
tgaattcgagctcggtacccggtgttttgcatgtgcattt

SEQ ID NO: 21 - DNA, 40 bp, synthetic construct
  misc_feature 1..40: note = Pn*_NCgl1064_R
  source 1..40: mol_type = other DNA
gtcgactctagaggatcccccacagccatacatgatgccg

SEQ ID NO: 22 - DNA, 40 bp, synthetic construct
  misc_feature 1..40: note = Pn*_NCgl0294_F
  source 1..40: mol_type = other DNA
tgaattcgagctcggtacccaactcacggccgtaggcgta

SEQ ID NO: 23 - DNA, 40 bp, synthetic construct
  misc_feature 1..40: note = Pn*_NCgl0294_R
  source 1..40: mol_type = other DNA
gtcgactctagaggatccccaccagtggctgcagctacgt

SEQ ID NO: 24 - DNA, 40 bp, synthetic construct
  misc_feature 1..40: note = Pn*_NCgl1720_F
  source 1..40: mol_type = other DNA
tgaattcgagctcggtacccagcaaccagtagtgaggtat

SEQ ID NO: 25 - DNA, 40 bp, synthetic construct
  misc_feature 1..40: note = Pn*_NCgl1720_R
  source 1..40: mol_type = other DNA
gtcgactctagaggatcccctccacaaagtggacagtgtt

SEQ ID NO: 26 - DNA, 40 bp, synthetic construct
  misc_feature 1..40: note = Pn*_NCgl0246_F
  source 1..40: mol_type = other DNA
tgaattcgagctcggtacccaggtgagctccttagggagc

SEQ ID NO: 27 - DNA, 40 bp, synthetic construct
  misc_feature 1..40: note = Pn*_NCgl0246_R
  source 1..40: mol_type = other DNA
gtcgactctagaggatccccttccgtggcgctcggtggtg

SEQ ID NO: 28 - DNA, 40 bp, synthetic construct
  misc_feature 1..40: note = Pn*_NCgl2356_F
  source 1..40: mol_type = other DNA
tgaattcgagctcggtacccccactgccatggctgccggt

SEQ ID NO: 29 - DNA, 40 bp, synthetic construct
  misc_feature 1..40: note = Pn*_NCgl2356_R
  source 1..40: mol_type = other DNA
gtcgactctagaggatccccgatgaggtgggtggagccaa

SEQ ID NO: 30 - DNA, 40 bp, synthetic construct
  misc_feature 1..40: note = Pn*_NCgl2521_F
  source 1..40: mol_type = other DNA
tgaattcgagctcggtacccgaggaaagcccaacgttggg

SEQ ID NO: 31 - DNA, 40 bp, synthetic construct
  misc_feature 1..40: note = Pn*_NCgl2521_R
  source 1..40: mol_type = other DNA
gtcgactctagaggatcccccgattccgcaccggctgcaa

SEQ ID NO: 32 - DNA, 40 bp, synthetic construct
  misc_feature 1..40: note = Pn*_NCgl2960_F
  source 1..40: mol_type = other DNA
tgaattcgagctcggtacccagtccttcattgccggggaa

SEQ ID NO: 33 - DNA, 40 bp, synthetic construct
  misc_feature 1..40: note = Pn*_NCgl2960_R
  source 1..40: mol_type = other DNA
gtcgactctagaggatcccccaaagcgtttgcgcttggat

SEQ ID NO: 34 - DNA, 16 bp, synthetic construct
  misc_feature 1..16: note = pNCgl0302_F
  source 1..16: mol_type = other DNA
acagcctgagcctgaa

SEQ ID NO: 35 - DNA, 16 bp, synthetic construct
  misc_feature 1..16: note = pNCgl0302_R
  source 1..16: mol_type = other DNA
agctgataacccaaag

SEQ ID NO: 36 - DNA, 16 bp, synthetic construct
  misc_feature 1..16: note = pNCgl0123_F
  source 1..16: mol_type = other DNA
caatggggtagtgggg

SEQ ID NO: 37 - DNA, 17 bp, synthetic construct
  misc_feature 1..17: note = pNCgl0123_R
  source 1..17: mol_type = other DNA
ccgtcttcgacaggaac

SEQ ID NO: 38 - DNA, 16 bp, synthetic construct
  misc_feature 1..16: note = pNCgl0625_F
  source 1..16: mol_type = other DNA
ttggtgaggcgggagt

SEQ ID NO: 39 - DNA, 16 bp, synthetic construct
  misc_feature 1..16: note = pNCgl0625_R
  source 1..16: mol_type = other DNA
accgccgcgataaccc

SEQ ID NO: 40 - DNA, 18 bp, synthetic construct
  misc_feature 1..18: note = pNCgl0276_F
  source 1..18: mol_type = other DNA
tgtttgttcgtggtgcag

SEQ ID NO: 41 - DNA, 18 bp, synthetic construct
  misc_feature 1..18: note = pNCgl0276_R
  source 1..18: mol_type = other DNA
cgccaaccttgccggtgg

SEQ ID NO: 42 - DNA, 17 bp, synthetic construct
  misc_feature 1..17: note = pNCgl1064_F
  source 1..17: mol_type = other DNA
tgtttgtccacaccacg

SEQ ID NO: 43 - DNA, 16 bp, synthetic construct
  misc_feature 1..16: note = pNCgl1064_R
  source 1..16: mol_type = other DNA
ccgccaacccagattt

SEQ ID NO: 44 - DNA, 16 bp, synthetic construct
  misc_feature 1..16: note = pNCgl0294_F
  source 1..16: mol_type = other DNA
gaggcttaattgcagg

SEQ ID NO: 45 - DNA, 16 bp, synthetic construct
  misc_feature 1..16: note = pNCgl0294_R
  source 1..16: mol_type = other DNA
cggtgaaaatgcctgg

SEQ ID NO: 46 - DNA, 18 bp, synthetic construct
  misc_feature 1..18: note = pNCgl1720_F
  source 1..18: mol_type = other DNA
cagaagagcttgatcatg

SEQ ID NO: 47 - DNA, 19 bp, synthetic construct
  misc_feature 1..19: note = pNCgl1720_R
  source 1..19: mol_type = other DNA
tgccgtcagcgtcaatcgg

SEQ ID NO: 48 - DNA, 18 bp, synthetic construct
  misc_feature 1..18: note = pNCgl0246_F
  source 1..18: mol_type = other DNA
gccagcatcgcggtactc

SEQ ID NO: 49 - DNA, 18 bp, synthetic construct
  misc_feature 1..18: note = pNCgl0246_R
  source 1..18: mol_type = other DNA
cagcaacaatgcagatct

SEQ ID NO: 50 - DNA, 15 bp, synthetic construct
  misc_feature 1..15: note = pNCgl2356_F
  source 1..15: mol_type = other DNA
gcggggcatcggatt

SEQ ID NO: 51 - DNA, 16 bp, synthetic construct
  misc_feature 1..16: note = pNCgl2356_R
  source 1..16: mol_type = other DNA
gtggtgggcgcgtgct

SEQ ID NO: 52 - DNA, 15 bp, synthetic construct
  misc_feature 1..15: note = pNCgl2521_F
  source 1..15: mol_type = other DNA
tagagaatcgagttg

SEQ ID NO: 53 - DNA, 16 bp, synthetic construct
  misc_feature 1..16: note = pNCgl2521_R
  source 1..16: mol_type = other DNA
tttccaggaccacaag

SEQ ID NO: 54 - DNA, 17 bp, synthetic construct
  misc_feature 1..17: note = pNCgl2960_F
  source 1..17: mol_type = other DNA
ttcggcggcgtcgagat

SEQ ID NO: 55 - DNA, 17 bp, synthetic construct
  misc_feature 1..17: note = pNCgl2960_R
  source 1..17: mol_type = other DNA
atttcggttaaggggta

SEQ ID NO: 56 - DNA, 170 bp, synthetic construct
  misc_feature 1..170: note = Wild type promoter of NCgl0302 gene
  source 1..170: mol_type = other DNA
actgcgcactgaaactgcgacctgggaacaagtctttcacgtttaaagcccaagcgatagtctattaggattagttttacgttttggcaggtcagtcccatttatacagcccagcgaaagggggtaaattcttgactacccccgattttgagagtgaaaagactcaagct

SEQ ID NO: 57 - DNA, 221 bp, synthetic construct
  misc_feature 1..221: note = Wild type promoter of NCgl0123 gene
  source 1..221: mol_type = other DNA
actttcacatcaaaaaaaagggggacaaatttctacatgaaattcgacgagatgaatgctattcattcttgtcttcagccacatctattcgaaatgaaatcctactgaatcaccagctagtccgcctaggtaaaaaaggcgtaattaacttatttatacataaaaacacaataaaaaccgcacacgcggcgaaacttcaataaatccctagactgcaaaaa

SEQ ID NO: 58 - DNA, 215 bp, synthetic construct
  misc_feature 1..215: note = Wild type promoter of NCgl0625 gene
  source 1..215: mol_type = other DNA
gagagatgatttataccatcctgcaccatttagagtggggctagtcatacccccataaccctagctgtacgcaatcgatttcaaatcagttggaaaaagtcaagaaaattacccgagaataaatttataccacacagtctattgcaatagaccaagctgttcagtagggtgcatgggagaagaatttcctaataaaaactcttaaggacctccaa

SEQ ID NO: 59 - DNA, 169 bp, synthetic construct
  misc_feature 1..169: note = Wild type promoter of NCgl0276 gene
  source 1..169: mol_type = other DNA
ggcgcaccccaggcgcaccccaggcgcaccccagcgcaccacaggcgcaccccagcgcaccacaggcgcaccagcccagcacaagagccaacgcaagtgtcaggcacgccagcaaaggggctagcaagaagcacgcccccgaagccttagaaatgcgttccccggtagg

SEQ ID NO: 60 - DNA, 57 bp, synthetic construct
  misc_feature 1..57: note = Wild type promoter of NCgl1064 gene
  source 1..57: mol_type = other DNA
cattttttaatcgaccgcttccatcatgttttaactaaggtttgtaggcttaaacct

SEQ ID NO: 61 - DNA, 306 bp, synthetic construct
  misc_feature 1..306: note = Wild type promoter of NCgl0294 gene
  source 1..306: mol_type = other DNA
gcgcctcggggggggtgtgcgcgggccgtcagtaacccggcaacggggggggattgtgccggggcaggccacactgtatatcggggccttgcacctgaaattatggcatatcaaacgccacaagacaacatcaaacccgattatttattcgaataacacgaatacttaacagtgtggcaaatgacacttcccgcacgccttctacattcccaatgcgcaaccccagcacgtcacttcaatctcattggtaactttagtttctttctcagtcttggaaagttgccaaaaagcgctaaactatgcggt

SEQ ID NO: 62 - DNA, 226 bp, synthetic construct
  misc_feature 1..226: note = Wild type promoter of NCgl1720 gene
  source 1..226: mol_type = other DNA
gcggttgattaaaaaaaaagaacactttgatatgaattaagtcgaagtgttcttttattaatttaaaagtatatttcagcaatggtaaatgaatctcataagttttaaagaaaagtattgcatttgtttgacaaggtgattatgcttcacattaatacttaataagaattgttctgggaagtaatataaaaagtcccgaacaaattagtgtgaaagggtttgtatc

SEQ ID NO: 63 - DNA, 246 bp, synthetic construct
  misc_feature 1..246: note = Wild type promoter of NCgl0246 gene
  source 1..246: mol_type = other DNA
ctttgtgcacctttcgatctacgtgctgacagttacccgctcaactctacctttataaactgtgtctacctagccagaggagtgttttctttctgcacagggttcctggggctttagcggatgcgtctcagccactgggacgcgttccaataaacagaccatatattgatattcgatttaatatttgagacaaaagtgacaggtgctacttcgcgagcaactctttagtcaactaccctgaatcaa

SEQ ID NO: 64 - DNA, 163 bp, synthetic construct
  misc_feature 1..163: note = Wild type promoter of NCgl2356 gene
  source 1..163: mol_type = other DNA
agattttgcttttcgacgctcccctccacctcattcaatgcggcggaggggatttccttgcatgttaagcctataggaaaaagtgtttgcatatcacccttgtattcgaacacgtgagcgggtagagtgggtggtaacaacacggggaaagggggaagacacc

SEQ ID NO: 65 - DNA, 198 bp, synthetic construct
  misc_feature 1..198: note = Wild type promoter of NCgl2521 gene
  source 1..198: mol_type = other DNA
gacgggctgaaaccaaaccagactgcccagcaacgacggaaatcccaaaagtgggcatccctgtttggtaccgagtacccacccgggcctgaaactccctggcaggcgggcgaagcgtggcaacaactggaatttaagagcacaattgaagtcgcaccaagttaggcaacacaatagccataacgttgaggagttcag

SEQ ID NO: 66 - DNA, 212 bp, synthetic construct
  misc_feature 1..212: note = Wild type promoter of NCgl2960 gene
  source 1..212: mol_type = other DNA
cctcaatgtttcacgtgaaacattgagggttttacacccaattaagaaaaaatgaattaaaccaaaacttcttaatcgcaggggttaaggtaagttcagctaatcaatgaaacttcccctttcagcccgttgaagaaccaatgagccctgcccgcacccagccccgagcggctttcctaaggaagctccgacccatcacatgtagcctttcc

SEQ ID NO: 67 - DNA, 5802 bp, synthetic construct
  misc_feature 1..5802: note = pDC24 vector
  source 1..5802: mol_type = other DNA
gttcgcttgctgtccataaaaccgcccagtctagctatcgccatgtaagcccactgcaagctacctgctttctctttgcgcttgcgttttcccttgtccagatagcccagtagctgacattcatccggggtcagcaccgtttctgcggactggctttctacgtgttccgcttcctttagcagcccttgcgccctgagtgcttgcggcagcgtgaagctagcttttatcgccattcgccattcaggctgcgcaactgttgggaagggcgatcggtgcgggcctcttcgctattacgccagctggcgaaagggggatgtgctgcaaggcgattaagttgggtaacgccagggttttcccagtcacgacgttgtaaaacgacggccagtgaattcgagctcggtacccggggatcctctagagtcgacctgcaggcatgcaagcttggcgtaatcatggtcatagctgtttcctgtgtgaaattgttatccgctcacaattccacacaacatacgagccggaagcataaagtgtaaagcctggggtgcctaatgagtgagctaactcacattaattgcgttgcgctcactgcccgctttccagtcgggaaacctgtcgtgccagctgcattaatgaatcggccaacgcgcggggagaggcggtttgcgtattgggcgctcttccgcttcctcgctcactgactcgctgcgctcggtcgttcggctgcggcgagcggtatcagctcactcaaaggcggtaatacggttatccacagaatcaggggataacgcaggaaagaacatgtgagcaaaaggccagcaaaaggccaggaaccgtaaaaaggccgcgttgctggcgtttttccataggctccgcccccctgacgagcatcacaaaaatcgacgctcaagtcagaggtggcgaaacccgacaggactataaagataccaggcgtttccccctggaagctccctcgtgcgctctcctgttccgaccctgccgcttaccggatacctgtccgcctttctcccttcgggaagcgtggcgctttctcaatgctcacgctgtaggtatctcagttcggtgtaggtcgttcgctccaagctgggctgtgtgcacgaaccccccgttcagcccgaccgctgcgccttatccggtaactatcgtcttgagtccaacccggtaagacacgacttatcgccactggcagcagccactggtaacaggattagcagagcgaggtatgtaggcggtgctacagagttcttgaagtggtggcctaactacggctacactagaaggacagtatttggtatctgcgctctgctgaagccagttaccttcggaaaaagagttggtagctcttgatccggcaaacaaaccaccgctggtagcggtggtttttttgtttgcaagcagcagattacgcgcagaaaaaaaggatctcaagaagatcctttgatcttttctacggggtctgacgctcagtggaacgaaaactcacgttaagggattttggtcatgagattatcaaaaaggatcttcacctagatccttttggggtgggcgaagaactccagcatgagatccccgcgctggaggatcatccagccctgatagaaacagaagccactggagcacctcaaaaacaccatcatacactaaatcagtaagttggcagcatcacccgacgcactttgcgccgaataaatacctgtgacggaagatcacttcgcagaataaataaatcctggtgtccctgttgataccgggaagccctgggccaacttttggcgaaaatgagacgttgatcggcacgtaagaggttccaactttcaccataatgaaataagatcactaccgggcgtattttttgagttatcgagattttcaggagctgatagaaacagaagccactggagcacctcaaaaacaccatcatacactaaatcagtaagttggcagcatcacccgacgcactttgcgccgaataaatacctgtgacggaagatcacttcgcagaataaataaatcctggtgtccctgttgataccgggaagccctgggccaacttttggcgaaaatgagacgttgatcggcacgtaagaggttccaactttcaccataatgaaataagatcactaccgggcgtattttttgagttatcgagattttcaggagctctttggcatcgtctctcgcctgtcccctcagttcagtaatttcctgcatttgcctgtttccagtcggtagatattccacaaaacagcagggaagcagcgcttttccgctgcataaccctgcttcggggtcattatagcgattttttcggtatatccatcctttttcgcacgatatacaggattttgccaaagggttcgtgtagactttccttggtgtatccaacggcgtcagccgggcaggataggtgaagtaggcccacccgcgagcgggtgttccttcttcactgtcccttattcgcacctggcggtgctcaacgggaatcctgctctgcgaggctggccggctaccgccggcgtaacagatgagggcaagcggatggctgatgaaaccaagccaaccaggaagggcagcccacctatcaaggtgtactgccttccagacgaacgaagagcgattgaggaaaaggcggcggcggccggcatgagcctgtcggcctacctgctggccgtcggccagggctacaaaatcacgggcgtcgtggactatgagcacgtccgcgagggcgtcccggaaaacgattccgaagcccaacctttcatagaaggcggcggtggaatcgaaatctcgtgatggcaggttgggcgtcgcttggtcggtcatttcgaaaaaggttaggaatacggttagccatttgcctgcttttatatagttcatatgggattcacctttatgttgataagaaataaaagaaaatgccaataggatatcggcattttcttttgcgtttttatttgttaactgttaattgtccttgttcaaggatgctgtctttgacaacagatgttttcttgcctttgatgttcagcaggaagctcggcgcaaacgttgattgtttgtctgcgtagaatcctctgtttgtcatatagcttgtaatcacgacattgtttcctttcgcttgaggtacagcgaagtgtgagtaagtaaaggttacatcgttaggcggatcaagatccatttttaacacaaggccagttttgttcagcggcttgtatgggccagttaaagaattagaaacataaccaagcatgtaaatatcgttagacgtaatgccgtcaatcgtcatttttgatccgcgggagtcagtgaacaggtaccatttgccgttcattttaaagacgttcgcgcgttcaatttcatctgttactgtgttagatgcaatcagcggtttcatcacttttttcagtgtgtaatcatcgtttagctcaatcataccgagagcgccgtttgctaactcagccgtgcgttttttatcgctttgcagaagtttttgactttcttgacggaagaatgatgtgcttttgccatagtatgctttgttaaataaagattcttcgccttggtagccatcttcagttccagtgtttgcttcaaatactaagtatttgtggcctttatcttctacgtagtgaggatctctcagcgtatggttgtcgcctgagctgtagttgccttcatcgatgaactgctgtacattttgatacgtttttccgtcaccgtcaaagattgatttataatcctctacaccgttgatgttcaaagagctgtctgatgctgatacgttaacttgtgcagttgtcagtgtttgtttgccgtaatgtttaccggagaaatcagtgtagaataaacggatttttccgtcagatgtaaatgtggctgaacctgaccattcttgtgtttggtcttttaggatagaatcatttgcatcgaatttgtcgctgtctttaaagacgcggccagcgtttttccagctgtcaatagaagtttcgccgactttttgatagaacatgtaaatcgatgtgtcatccgcatttttaggatctccggctaatgcaaagacgatgtggtagccgtgatagtttgcgacagtgccgtcagcgttttgtaatggccagctgtcccaaacgtccaggccttttgcagaagagatatttttaattgtggacgaatcaaattcagaaacttgatatttttcatttttttgctgttcagggatttgcagcatatcatggcgtgtaatatgggaaatgccgtatgtttccttatatggcttttggttcgtttctttcgcaaacgcttgagttgcgcctcctgccagcagtgcggtagtaaaggttaatactgttgcttgttttgcaaactttttgatgttcatcgttcatgtctccttttttatgtactgtgttagcggtctgcttcttccagccctcctgtttgaagatggcaagttagttacgcacaataaaaaaagacctaaaatatgtaaggggtgacgccaaagtatacactttgccctttacacattttaggtcttgcctgctttatcagtaacaaacccgcgcgatttacttttcgacctcattctattagactctcgtttggattgcaactggtctattttcctcttttgtttgatagaaaatcataaaaggatttgcagactacgggcctaaagaactaaaaaatctatctgtttcttttcattctctgtattttttatagtttctgttgcatgggcataaagttgcctttttaatcacaattcagaaaatatcataatatctcatttcactaaataatagtgaacggcaggtatatgtgatgggttaaaaaggatcaccccagagtcccgctcagaagaactcgtcaagaaggcgatagaaggcgatgcgctgcgaatcgggagcggcgataccgtaaagcacgaggaagcggtcagcccattcgccgccaagctcttcagcaatatcacgggtagccaacgctatgtcctgatagcggtccgccacacccagccggccacagtcgatgaatccagaaaagcggccattttccaccatgatattcggcaagcaggcatcgccatgggtcacgacgagatcctcgccgtcgggcatccgcgccttgagcctggcgaacagttcggctggcgcgagcccctgatgctcttcgtccagatcatcctgatcgacaagaccggcttccatccgagtacgtgctcgctcgatgcgatgtttcgcttggtggtcgaatgggcaggtagccggatcaagcgtatgcagccgccgcattgcatcagccatgatggatactttctcggcaggagcaaggtgagatgacaggagatcctgccccggcacttcgcccaatagcagccagtcccttcccgcttcagtgacaacgtcgagacagctgcgcaaggaacgcccgtcgtggccagccacgatagccgcgctgcctcgtcttggagttcattcagggcaccggacaggtcggtcttgacaaaaagaaccgggcgcccctgcgctgacagccggaacacggcggcatcagagcagccgattgtctgttgtgcccagtcatagccgaatagcctctccacccaagcggccggagaacctgcgtgcaatccatcttgttcaatcatgcgaaacgatcctcatcctgtctcttgatcagatcttgatcccctgcgccatcagatccttggcggcaagaaagccatccagtttactttgcagggcttcccaaccttaccagagggcgccccagctggcaattccg